European Patent Application EP 4 253 417 A1, published October 4, 2023. Title: Novel anti-C-MPL antibodies and uses thereof. Applicant: Daegu Gyeongbuk Institute of Science and Technology KOSIN UNIVERSITY INDUSTRY-ACADEMY COOPERATION Inje university industry-academic cooperation foundation. The sequence listing filed with the application follows.

SEQUENCE LISTING (6 sequences)

SEQ ID NO: 1 - protein, 8 aa, Artificial Sequence
  VH CDR1
RDTFNTYG

SEQ ID NO: 2 - protein, 8 aa, Artificial Sequence
  VH CDR2
IIPIFGTA

SEQ ID NO: 3 - protein, 11 aa, Artificial Sequence
  VH CDR3
ARDRRAGGYDY

SEQ ID NO: 4 - protein, 6 aa, Artificial Sequence
  VL CDR1
QGLGRW

SEQ ID NO: 5 - protein, 3 aa, Artificial Sequence
  VL CDR2
AAS

SEQ ID NO: 6 - protein, 9 aa, Artificial Sequence
  VL CDR3
QQSNSFPWT